European Patent Specification EP 3 534 963 B1, published April 17, 2024. Title: Formulations of Pegylated Arginine Deiminase. Applicant: Polaris Group Wu, Bor-Wen Thomson, James Tsai, Wen-Chin. Application PCT/US2017/059732. The sequence listing filed with the application follows.

SEQUENCE LISTING (56 sequences)

SEQ ID NO: 1 - protein, 409 aa, Mycoplasma hominis
MSVFDSKFNGIHVYSEIGELETVLVHEPGREIDYITPARLDELLFSAILESHDARKEHQSFVKIMKDRGINVVELTDLVAETYDLASKAAKEEFIETFLEETVPVLTEANKKAVRAFLLSKPTHEMVEFMMSGITKYELGVESENELIVDPMPNLYFTRDPFASVGNGVTIHFMRYIVRRRETLFARFVFRNHPKLVKTPWYYDPAMKMPIEGGDVFIYNNETLVVGVSERTDLDTITLLAKNIKANKEVEFKRIVAINVPKWTNLMHLDTWLTMLDKNKFLYSPIANDVFKFWDYDLVNGGAEPQPQLNGLPLDKLLASIINKEPVLIPIGGAGATEMEIARETNFDGTNYLAIKPGLVIGYDRNEKTNAALKAAGITVLPFHGNQLSLGMGNARCMSMPLSRKDVKW

SEQ ID NO: 2 - protein, 409 aa, Artificial Sequence
  Mutated arginine deaminase
MSVFDSKFNGIHVYSEIGELETVLVHEPGREIDYITPARLDELLFSAILESHDARKEHQSFVKIMKDRGINVVELTDLVAETYDLASKAAKEEFIETFLEETVPVLTEANKEAVRAFLLSKPTHEMVEFMMSGITKYELGVESENELIVDPMPNLYFTRDPFASVGNGVTIHFMRYIVRRRETLFARFVFRNHPKLVKTPWYYDPAMKMSIEGGDVFIYNNETLVVGVSERTDLDTITLLAKNIKANKEVEFKRIVAINVPKWTNLMHLDTWLTMLDKNKFLYSPIANDVFKFWDYDLVNGGAEPQPQLNGLPLDKLLASIINKEPVLIPIGGAGATEMEIARETNFDGTNYLAIKPGLVIGYDRNEKTNAALKAAGITVLPFHGNQLSLGMGNARCMSMPLSRKDVKW

SEQ ID NO: 3 - protein, 392 aa, Mycoplasma phocicerebrale
IHVYSEIGELETVLVHEPGREIDYITPARLDELLFSAILESHDARKEHQSFVKQLKDNGINVVELTDLVAETFDLASKEEQEKLIEEFLEDSEPVLSEAHKTAVRKFLTSRKSTREMVEFMMAGITKYDLGIEADHELIVDPMPNLYFTRDPFASVGNGVTIHYMRYKVRQRETLFSRFVFSNHPKLVKTPWYYDPAMKMSIEGGDVFIYNNDTLVVGVSERTDLETITLLAKNIKANKEVEFKRIVAINVPKWTNLMHLDTWLTMLDKDKFLYSPIANDVFKFWDYDLVNGGAEPQPKENGLPLEGLLQSIINKKPVLIPIAGNNASHIDIERETHFDGTNYLAIKPGVVIGYARNEKTNAALAAAGIKVLPFHGNQLSLGMGNARCMSMP

SEQ ID NO: 4 - protein, 410 aa, Mycoplasma arginini
MSVFDSKFKGIHVYSEIGELESVLVHEPGREIDYITPARLDELLFSAILESHDARKEHKQFVAELKANDINVVELIDLVAETYDLASQEAKDKLIEEFLEDSEPVLSEEHKVVVRNFLKAKKTSRELVEIMMAGITKYDLGIEADHELIVDPMPNLYFTRDPFASVGNGVTIHYMRYKVRQRETLFSRFVFSNHPKLINTPWYYDPSLKLSIEGGDVFIYNNDTLVVGVSERTDLQTVTLLAKNIVANKECEFKRIVAINVPKWTNLMHLDTWLTMLDKDKFLYSPIANDVFKFWDYDLVNGGAEPQPVENGLPLEGLLQSIINKKPVLIPIAGEGASQMEIERETHFDGTNYLAIRPGVVIGYSRNEKTNAALEAAGIKVLPFHGNQLSLGMGNARCMSMPLSRKDVKW

SEQ ID NO: 5 - protein, 409 aa, Mycoplasma arthritidis
MSVFDSKFKGIHVYSEIGELETVLVHEPGKEIDYITPARLDELLFSAILESHDARKEHKEFVAELKKRGINVVELVDLIVETYDLASKEAKEKLLEEFLDDSVPVLSDEHRAAVKKFLQSQKSTRSLVEYMIAGITKHDLKIESDLELIVDPMPNLYFTRDPFASVGNGVTIHYMRYKVRQRETLFSRFVFSNHPKLVNTPWYYDPAEGLSIEGGDVFIYNNDTLVVGVSERTDLQTITLLAKNIKANKECEFKRIVAINVPKWTNLMHLDTWLTMLDKDKFLYSPIANDVFKFWDYDLVNGGDAPQPVDNGLPLEDLLKSIIGKKPTLIPIAGAGASQIDIERETHFDGTNYLAVAPGIVIGYARNEKTNAALEAAGITVLPFRGNQLSLGMGNARCMSMPLSRKDVK

SEQ ID NO: 6 - protein, 408 aa, Mycoplasma orale
  misc_feature (201)..(201): Xaa can be any naturally occurring amino acid
  misc_feature (263)..(263): Xaa can be any naturally occurring amino acid
  misc_feature (272)..(272): Xaa can be any naturally occurring amino acid
  misc_feature (294)..(294): Xaa can be any naturally occurring amino acid
SVFSDKFNGIHVYSEIGDLESVLVHEPGKEIDYITPARLDELLFSAILESTDARKEHKEFVEILKKQGINVVELVDLVVETYNLVDKKTQEKLLKDFLDDSEPVLSPEHRKAVEKFLKSLKSTKELIQYMMAGITKYDLGIKADKELIVDPMPNLYFTRDPFASVGNGVTIHYMRYKVRQRETLFSKFIFTNHPKLVKTPXYYDPAMKLSIEGGDVFIYNNDTLVVGVSERTDLETITLLAKNIKANKECEFKRIVAINVPKXTNLMHLDTXLTMLDKDKFLYSPIANDVFKFXDYDLVNGGSNPEPVVNGLPLDKLLESIINKKPVLIPIAGKGATEIETAVETHFDGTNYLAIKPGVVVGYSRNVKTNAALEANGIKVLPFKGNQLSLGMGNARCMSMPLSRKDVK

SEQ ID NO: 7 - protein, 391 aa, Mycoplasma gateae
IHVYSEIGELESVLVHEPGREIDYITPARLDELLFSAILESHDARKEHKLFVSELKANDINVVELTDLVTETYDLASQEAKDNLIEEFLEDSEPVLTEELKSVVRTYLKSIKSTRELIQMMMAGITKYDLGIEADHELIVDPMPNLYFTRDPFASVGNGVTIHYMRYKVRQRETLFSRFVFSNHPKLVNTPWYYDPSLKLSIEGGDVFIYNNNTLVVGVSERTDLETVTLLAKNIVANKECEFKRIVAINVPKWTNLMHLDTWLTMLDKDKFLYSPIANDVFKFWDYDLVNGGEEPQPVENGLPLEGLLESIINKKPILIPIAGEGASQIDIERETHFDGTNYLAIRPGVVIGYSRNEKTNAALEAAGIKVLPFHGNQLSLGMGNARCMSM

SEQ ID NO: 8 - protein, 392 aa, Mycoplasma phocidae
IHVYSEIGELQTVLVHEPGREIEYITPARLDELLFSAILESHDARKEHQEFVAELKKNNINVVELTDLVSETYDMVSKEKQEKLIEEFLEDSEPVLSEEHKGLVRKFLKSLKSSKELIQYMMAGITKHDLNIEADHELIVDPMPNLYFTRDPFASVGNGVTIHYMRYKVRQRETLFSRFIFANHPKLMNTPLYYNPDMKLSIEGGDVFVYNNETLVVGVSERTDLDTITLLAKNIKANKEREFKRIVAINVPKWTNLMHLDTWLTMLDKDKFLYSPIANDVFKFWDYDLVNGGDEPQPKVNGLPLEKLLESIINKKPILIPIAGTSASNIDVERETHFDGTNYLAIAPGVVIGYSRNVKTNEALEAAGIKVLPFKGNQLSLGMGNARCMSMP

SEQ ID NO: 9 - protein, 401 aa, Mycoplasma columbinum
MSKINVYSEIGELKEVLVHTPGDEIRRISPSRLDELLFSAILEPNEAIKEHKGFLKILQDKGIKVIQLSDLVAETYTYHATQKEREAFIEKWLDEAEPALTKDLRAKVKSYVLSKEGTPVAMVRTMMAGVSKQELNVESETELVVDPMPNLYFTRDPFASAGNGISLNNMKYVTRKRETIFAEFIFATHPDYKTTPHWFDRLDEGNIEGGDVFIYNKDTLVIGVSERTNKEAILTIAKKIKNNKEAKFKKIVAINVPPMPNLMHLDTWLTMVDKDKFLYSPNMLSVLKVWEIDLSKEIEMVETNKPLADVLESIIGVKPVLIPIAGKGATQLDIDIETHFDGTNYLTIAPGVVVGYSRNIKTEAALRAAGVTVLSFEGNQLSLGMGSARCMSMPLVREDVK

SEQ ID NO: 10 - protein, 407 aa, Mycoplasma iowae
MGNNIPKKINVFSEIGNLKRVLVHTPGKEIEYVTPQRLDELLFSAILDPVRAREEHKEFIKILESQGVEVVQLVDLTAETYDVAESQAKENFIQKWLDESLPKLTDENRNKVYSLLKSLEKDPKEMIRKMMSGVLASEIGVKSDVELIVDPMPNLYFTRDPFASVGNGITLHRMFRPTRRRETIFADFIFSNHPEYKSTQKYYEREDKFSLEGGDVFIYNNKTLVVGVSERTEKGAIKALAKAVQNNSNMSFEKIYAINVPKMSNLMHLDTWLTMLDTDKFLYSPNMMGVLKIWEIDLSDKSLKWKEIRDSLDHFLSTIIGKKAITVPVAGKDAMQFEIDIETHFDATNFIAVAPGVVIGYDRNKKTNEALKEAGIKVLSWNGDQLSLGMGSARCMTMPLYREELKK

SEQ ID NO: 11 - protein, 402 aa, Mycoplasma crocodyli
MNKINVYSEVGKLKEVLVHTPGDEIRRISPSRLEELLFSAILEPDSAIEEHKRFLKILEDNNIKVIQLDQLVADTYELVNPSVRDAFIEKWLNESEPKLDKKLREKVKEYLLHTQKTVGTKRMVRIMMAGVDRVELGVELDRQLVVDPMPNLYFTRDPFASAGNGISLNNMKYVTRKRETIFSEFIFENHPDYKTTPHWFDRLDKGNIEGGDVFIYNRTTLVIGISERTNKDALLTIANNIKSNKESKFERIVAVNVPPMPNLMHLDTWLTMVDHDKFLYSPNMMKTLKFWTIDLTKPIKMVELEESLSDMIETIIGKKPVLIPIAGHDASPLDVDIETHFDGTNYLTIAPGVVVGYSRNKLTEKALTKAGVKVLSFEGNQLSLGMGSARCMSMPLVREDIK

SEQ ID NO: 12 - protein, 430 aa, Mycoplasma fermentans
MQIIAKIDLLTNMLIFMKIYFIGRLIMKKINVYSEYGKLKEVLVHTPGDEIRRIAPSRLDELLFSAILEPDSAIAEHKRFVQLLKDNGIKVIQLDELFAKTFDLVSESVKQSLIERWLDECEPKLDATLRAKVKEYILELKAKSSKKMVRVMMAGIDKKELGIELDRDLVVDPMPNLYFTRDPFASVGNGISLHHMKYVTRQRETIFSEFIFDNNLDYNTVPRWFDRKDEGRIEGGDVFIYSADTLVVGVSERTNKEAINVMARKIAADKEVKFKRIYAINVPPMPNLMHLDTWLTMLDKNKFLYSPNMLSVLKVWRIDLNDPDFVWHEIEGSLEEILEQIIGMKPILIPIAGKGASQLDIDIETHFDGTNYLTIAPSVVVGYSRNEKTEKALKAAKVKVLSFEGNQLSLGMGSARCMSMPLIREDIKKK

SEQ ID NO: 13 - protein, 452 aa, Mycoplasma penetrans
MVITIALNILNKIYFKPQNRSILKLYRLPSLCTQISIFIGGKMSSIDKNSLGNGINVYSEIGELKEVLVHTPGDEIRYTAPSRLEELLFSAVLKADTAIEEHKGFVKILQNNGIKVIQLCDLVAETYELCSKEVRNSFIEQYLDEALPVLKKEIRPVVKDYLLSFPTVQMVRKMMSGILANELNIKQDNPLIIDGMPNLYFTRDPFASMGNGVSINCMKYPTRKREVIFSRFVFTNNPKYKNTPRYFDIVGNNGTIEGGDIFIYNSKTLVIGNSERTNFAAIESVAKNIQANKDCTFERIVVINVPPMPNLMHLDTWLTMLDYDKFLYSPNMMNVLKIWEIDLNVKPVKFVEKKGTLEEVLYSIIDKKPILIPIAGKGANQLDIDIETHFDGTNYLTIAPGVVVGYERNEKTQKALVEAGIKVLSFNGSQLSLGMGSARCMSMPLIRENLKK

SEQ ID NO: 14 - protein, 403 aa, Mycoplasma gallisepticum
MFNKIRVYSEIGKLRKVLVHTPGKELDYVTPQRLDELLFSSLLNPIKARQEHETFIKLLEDHDVECVQLSTLTAQTFQAVNSKIQEEFINRWLDECLPVLSEINRLKVYDYLKSLATNPQVMIRKMMSGILAKEVGIQSEVELVADPMPNLYFTRDPFASIGKGITLHSMFHPTRKRETIFADFIFSHHPEYKNAPKYYSREDKYSIEGGDLFVYDDKTLVIGVSERTEKKAIQSLAEKLRQNDETSFEKIYAINVPKMSNLMHLDTWLTMLDYDKFLYSPNMMGVLKIWEIDLIHPTLIWRELNESLEGFLSMVIGKKATLIPVAGEDSTQIEIDVETNFDATNFLVIQPGVVVGYDRNYKTNQALRDAGVKVISWNGDQLSLGMGSARCMSMPLYRDPIKK

SEQ ID NO: 15 - protein, 402 aa, Mycoplasma alligatoris
MSKINVYSEVGRLKEVLVHTPGDEIRRISPTRLEELLFSAILEPDTAIEEHKRFLNVLEKNGIKAIQLDELVAQTYDQVDQKIKDEFIDQWLQEAKPVLNDQLKKLVKNYLLKSQKEFSTKKMVRIMMAGIDKKEINIDLDRDLVVDPMPNLYFTRDPFASVGNGISLHNMKYQTRKRETIFAQFIFKYNKDYKTTPHWFDRFDHGSIEGGDVFVYTKDTLVIGISERTTKEAVLNIAKKIKANTDSKFKKIVAINVPPMPNLMHLDTWITMVDHDKFLYSPNMMKSLKFWLIDLSKEIKMVELEESLSNMLEAIIGKKPILIPIAGKNASQLDIDIETHFDGTNYLTIAPGVVVGYSRNKLTQKALEDAGVKVLSFDGNQLSLGMGSARCMSMPLVREDIK

SEQ ID NO: 16 - protein, 438 aa, Mycoplasma pneumoniae
MSKKQLVKTDGHNQLDQPNTKALQLKKKQFNSGVRVTSEISFLREVIAHHPGIETERVIDNQTFGSAMYLERAQKEHQLFIKILRQHGTKVHYLQDLLLEALSAADPNVRQDFIKNFLLESGIKSVSTFEACLNFFRSLDSLVDVIKVMFGGIKVSDVPPITPQRFADIHVSNSPFLIKPLSFSLYPHKFFNTLGTGVALFVTNDSELKRHSLVYEYIMRFHPRFDGVKLYTNRDFKNCLINSSDIIQISNEILLIGISHDTDVLGIESLARNLLSDHTNPIKQIIAINIHKFGAKTNLNKLIAMVDVDKFIIARKVLQATEIFELTATAQRDVDGLAQIKFKPLKFNFGEIIEAIIDKQPRFVIIGGGDEVAERKELLDCGMGVLNLSPGEIVVFDRNHYTNNLLNELGLIIHKIPASELSRGPSGPLEMVCSLWRE

SEQ ID NO: 17 - protein, 409 aa, Mycoplasma mobile
MKDTKDIINVFSEIGELKKVLIHTPGNELKYVSPYRLDELLFSNVLEWREAKKEHNEFIQKLKSEGVEPVELTDLVAESFEESSIKVKNDFIRQYLDEATPILDGLTKQKLLPFFLDIKHSTRKTIELMMSGITQKDISISHIERELIIDPMPNLYFSRDNFISIGNSVIISNMKYKTRKRETIFTDFIFKNHPLYKKVNMAFERKDLNNQISIIEGGDVLVYSKEILIIGISERTTMSAILELAENFKKTKRSFKKIYGVEVPKMKNLMHLDTWLTMIDYDKFIYSPNVLTDLKFWEINLDYEKISSKELHASLSEFLKLIIGKDPILIPIGGKGASQITIDIETNFVAANYLVIRPGVVIGYSRNYETQKALEGHGVKVIAFEGNQLSLGMGSSRCMSMPLIRSNLK

SEQ ID NO: 18 - protein, 411 aa, Streptococcus pyogenes
MTAQTPIHVYSEIGKLKKVLLHRPGKEIENLMPDYLERLLFDDIPFLEDAQKEHDAFAQALRDEGIEVLYLETLAAESLVTPEIREAFIDEYLSEANIRGRATKKAIRELLMAIEDNQELIEKTMAGVQKSELPEIPASEKGLTDLVESNYPFAIDPMPNLYFTRDPFATIGTGVSLNHMFSETRNRETLYGKYIFTHHPIYGGGKVPMVYDRNETTRIEGGDELVLSKDVLAVGISQRTDAASIEKLLVNIFKQNLGFKKVLAFEFANNRKFMHLDTVFTMVDYDKFTIHPEIEGDLRVYSVTYDNEELHIVEEKGDLAELLAANLGVEKVDLIRCGGDNLVAAGREQWNDGSNTLTIAPGVVVVYNRNTITNAILESKGLKLIKIHGSELVRGRGGPRCMSMPFEREDI

SEQ ID NO: 19 - protein, 408 aa, Enterococcus faecalis
MSHPINVFSEIGKLKTVMLHRPGKELENLMPDYLERLLFDDIPFLEKAQAEHDAFAELLRSKDIEVVYLEDLAAEALINEEVRRQFIDQFLEEANIRSESAKEKVRELMLEIDDNEELIQKAIAGIQKQELPKYEQEFLTDMVEADYPFIIDPMPNLYFTRDNFATMGHGISLNHMYSVTRQRETIFGQYIFDYHPRFAGKEVPRVYDRSESTRIEGGDELILSKEVVAIGISQRTDAASIEKIARNIFEQKLGFKNILAFDIGEHRKFMHLDTVFTMIDYDKFTIHPEIEGGLVVYSITEKADGDIQITKEKDTLDNILCKYLHLDNVQLIRCGAGNLTAAAREQWNDGSNTLAIAPGEVVVYDRNTITNKALEEAGVKLNYIPGSELVRGRGGPRCMSMPLYREDL

SEQ ID NO: 20 - protein, 403 aa, Mycoplasma capricolum
MEKKINVFSEIGTLKTVLVHRPGDEIENLTPELLERLLFDDVPFKDVAVKEHDAFTKIMRDNGVEVLYIEKLAAETLDQHPDLREKFIDQFISEANIEDKYKEKYRDFISSLDNYRMIKKMIAGTKKLELGIDEGYKAYPFIADPLPNVLFQRDPFSSVGFGITMNRMWSVTRNRETIFPDLVFKHHNRFANQVPYYYERDWKEETIEGGDILVLNKETLIIGVTQRTTLKAIEKFSERLFNDPESSYSKVIALDLPKSRAFMHLDTVFTNIDYDKFIAHPLIFDCIDEFKIYEVSKQGTKEVKKTLIELLSDAAGREVQIIRCGGNDVVGASREQWNDGTNVVALRPGKVIAYERNWITIDLLRKAGVEVLTIASSELSRGRGGPRCMTMPLWREDLQEIKR

SEQ ID NO: 21 - protein, 410 aa, Halothermothrix orenii
MFKKSPLNVTSEIGKLKKVLLHRPGHEIENLTPDLLERLLFDDIPYLKVAQEEHDAFAQTLRDNGVEVLYLHELAAEAIQEDEIRKKFIEQFLDEAGVIGKGARQVLKEYFADMDNETLIRKMMAGVRKKEIPAIEKVASLNDMVEEDYPFVLDPMPNLYFTRDPFATIGTGITLNHMRTETRNREVIFAEYIFSYHPDFKDTEIPFWFDRNETTSIEGGDELILSDKVLAMGISERTDAASIEKVARNIFTDGQPFETILAFKIPEKRAFMHLDTVFTMVDYDKFTIHAEIEGPLKVYSITKGDNDELKIDEEKATLEDTLKKYLGLDEVTLIRCAGGDYIDAGREQWNDGSNTLAIAPGEVVVYNRNHTTNRLLEEHGIKLHVIPSSELSRGRGGPRCMSMPLVREDI

SEQ ID NO: 22 - protein, 411 aa, Staphylococcus aureus
MTDGPIKVNSEIGALKTVLLKRPGKELENLVPDYLDGLLFDDIPYLEVAQKEHDHFAQVLREEGVEVLYLEKLAAESIENPQVRSEFIDDVLAESKKTILGHEEEIKALFATLSNQELVDKIMSGVRKEEINPKCTHLVEYMDDKYPFYLDPMPNLYFTRDPQASIGHGITINRMFWRARRRESIFIQYIVKHHPRFKDANIPIWLDRDCPFNIEGGDELVLSKDVLAIGVSERTSAQAIEKLARRIFENPQATFKKVVAIEIPTSRTFMHLDTVFTMIDYDKFTMHSAILKAEGNMNIFIIEYDDVNKDIAIKQSSHLKDTLEDVLGIDDIQFIPTGNGDVIDGAREQWNDGSNTLCIRPGVVVTYDRNYVSNDLLRQKGIKVIEISGSELVRGRGGPRCMSQPLFREDI

SEQ ID NO: 23 - protein, 417 aa, Pseudomonas plecoglossicida
MSAEKQKYGVHSEAGKLRKVMVCAPGLAHKRLTPSNCDELLFDDVIWVDQAKRDHFDFVTKMRERGVDVLEMHNLLTDIVQNPEALKWILDRKITPDTVGVGLTNEVRSWLEGQEPRHLAEFLIGGVAGQDLPESEGASVVKMYNDYLGHSSFILPPLPNTQFTRDTTCWIYGGVTLNPMYWPARRQETLLTTAIYKFHPEFTKADFQVWYGDPDQEHGQATLEGGDVMPIGKGIVLIGMGERTSRQAIGQLAQNLFAKGAVEQVIVAGLPKSRAAMHLDTVFSFCDRDLVTVFPEVVREIVPFIIRPDESKPYGMDVRRENKSFIEVVGEQLGVKLRVVETGGNSFAAEREQWDDGNNVVALEPGVVIGYDRNTYTNTLLRKAGIEVITISAGELGRGRGGGHCMTCPIVRDPINY

SEQ ID NO: 24 - protein, 417 aa, Pseudomonas putida
MSAEKQKYGVHSEAGKLRKVMVCAPGLAHKRLTPSNCDELLFDDVIWVDQAKRDHFDFVTKMRERGVDVLEMHNLLTDIVQNKDALKWILDRKITPDTVGVGLTNEVRSWLEGLEPRHLAEFLIGGVAGQDLPQSEGADVVKMYNDYLGHSSFILPPLPNTQFTRDTTCWIYGGVTLNPMYWPARRQETLLTTAIYKFHPQFTGADFQVWYGDPDKDHGNATLEGGDVMPIGKGIVLIGMGERTSRQAIGQLAQNLFAKGAVEKVIVAGLPKSRAAMHLDTVFSFCDRDLVTIFPEVVKEIVPFIIRPDESKPYGMDVRRENKSFIEVVGEQLGVKLRVVETGGNSFAAEREQWDDGNNVVAVEPGVVIGYDRNTYTNTLLRKAGIEVITISAGELGRGRGGGHCMTCPIVRDPIDY

SEQ ID NO: 25 - protein, 418 aa, Pseudomonas aeruginosa
MSTEKTKLGVHSEAGKLRKVMVCSPGLAHQRLTPSNCDELLFDDVIWVNQAKRDHFDFVTKMRERGIDVLEMHNLLTETIQNPEALKWILDRKITADSVGLGLTSELRSWLESLEPRKLAEYLIGGVAADDLPASEGANILKMYREYLGHSSFLLPPLPNTQFTRDTTCWIYGGVTLNPMYWPARRQETLLTTAIYKFHPEFANAEFEIWYGDPDKDHGSSTLEGGDVMPIGNGVVLIGMGERSSRQAIGQVAQSLFAKGAAERVIVAGLPKSRAAMHLDTVFSFCDRDLVTVFPEVVKEIVPFSLRPDASSPYGMSIRREEKTFLEVVAESLGLKKLRVVETGGNSFAAEREQWDDGNNVVCLEPGVVVGYDRNTYTNTLLRKAGVEVITISASELGRGRGGGHCMTCPIIRDPIDY

SEQ ID NO: 26 - protein, 402 aa, Mycobacterium tuberculosis complex
MGVELGSNSEVGALRVVILHRPGAELRRLTPRNTDQLLFDGLPWVSRAQDEHDEFAELLASRGAEVLLLSDLLTEALHHSGAARMQGIAAAVDAPRLGLPLAQELSAYLRSLDPGRLAHVLTAGMTFNELPSDTRTDVSLVLRMHHGGDFVIEPLPNLVFTRDSSIWIGPRVVIPSLALRARVREASLTDLIYAHHPRFTGVRRAYESRTAPVEGGDVLLLAPGVVAVGVGERTTPAGAEALARSLFDDDLAHTVLAVPIAQQRAQMHLDTVCTMVDTDTMVMYANVVDTLEAFTIQRTPDGVTIGDAAPFAEAAAKAMGIDKLRVIHTGMDPVVAEREQWDDGNNTLALAPGVVVAYERNVQTNARLQDAGIEVLTIAGSELGTGRGGPRCMSCPAARDPL

SEQ ID NO: 27 - protein, 409 aa, Mycoplasma arthritidis; identical to SEQ ID NO: 5

SEQ ID NO: 28 - protein, 410 aa, Artificial Sequence
  Artificial full length of Mycoplasma phocicerebrale
MSVFDSKFNGIHVYSEIGELETVLVHEPGREIDYITPARLDELLFSAILESHDARKEHQSFVKQLKDNGINVVELTDLVAETFDLASKEEQEKLIEEFLEDSEPVLSEAHKTAVRKFLTSRKSTREMVEFMMAGITKYDLGIEADHELIVDPMPNLYFTRDPFASVGNGVTIHYMRYKVRQRETLFSRFVFSNHPKLVKTPWYYDPAMKMSIEGGDVFIYNNDTLVVGVSERTDLETITLLAKNIKANKEVEFKRIVAINVPKWTNLMHLDTWLTMLDKDKFLYSPIANDVFKFWDYDLVNGGAEPQPKENGLPLEGLLQSIINKKPVLIPIAGNNASHIDIERETHFDGTNYLAIKPGVVIGYARNEKTNAALAAAGIKVLPFHGNQLSLGMGNARCMSMPLSRKDVKW

SEQ ID NO: 29 - protein, 410 aa, Artificial Sequence
  Artificial full length of Mycoplasma gateae
MSVFDSKFNGIHVYSEIGELESVLVHEPGREIDYITPARLDELLFSAILESHDARKEHKLFVSELKANDINVVELTDLVTETYDLASQEAKDNLIEEFLEDSEPVLTEELKSVVRTYLKSIKSTRELIQMMMAGITKYDLGIEADHELIVDPMPNLYFTRDPFASVGNGVTIHYMRYKVRQRETLFSRFVFSNHPKLVNTPWYYDPSLKLSIEGGDVFIYNNNTLVVGVSERTDLETVTLLAKNIVANKECEFKRIVAINVPKWTNLMHLDTWLTMLDKDKFLYSPIANDVFKFWDYDLVNGGEEPQPVENGLPLEGLLESIINKKPILIPIAGEGASQIDIERETHFDGTNYLAIRPGVVIGYSRNEKTNAALEAAGIKVLPFHGNQLSLGMGNARCMSMPLSRKDVKW

SEQ ID NO: 30 - protein, 410 aa, Artificial Sequence
  Artificial full length of Mycoplasma phocidae
MSVFDSKFNGIHVYSEIGELQTVLVHEPGREIEYITPARLDELLFSAILESHDARKEHQEFVAELKKNNINVVELTDLVSETYDMVSKEKQEKLIEEFLEDSEPVLSEEHKGLVRKFLKSLKSSKELIQYMMAGITKHDLNIEADHELIVDPMPNLYFTRDPFASVGNGVTIHYMRYKVRQRETLFSRFIFANHPKLMNTPLYYNPDMKLSIEGGDVFVYNNETLVVGVSERTDLDTITLLAKNIKANKEREFKRIVAINVPKWTNLMHLDTWLTMLDKDKFLYSPIANDVFKFWDYDLVNGGDEPQPKVNGLPLEKLLESIINKKPILIPIAGTSASNIDVERETHFDGTNYLAIAPGVVIGYSRNVKTNEALEAAGIKVLPFKGNQLSLGMGNARCMSMPLSRKDVKW

SEQ ID NO: 31 - protein, 410 aa, Mycoplasma salivarium
MSVFSSKFNGIHVYSEIGELETVLVHEPGKEIDYITPSRLDELLFSAILESHDARKEHQEFVATLKKEKINVVELTDLVTETYDLVDQKTKDKLIDEFLEDSEPVLTAELKATVKKFLKSFKETRKLIEVMMAGITKYDLGIKADRELIVDPMPNLYFTRDPFASVGNGVTIHYMRYKVRQRETLFSRFIFNNHPKLVKTPWYYDPAMKMSIEGGDVFIYNNDTLVVGVSERTDLDTITLLAKNIKANKECEFKRIVAINVPKWTNLMHLDTWLTMLDKDKFLYSPIANDIFKFWDYDLVNGGANPQPKDNGLPLDKLLKSIIGKEPVLIPIAGHHATEIEVARETHFDGTNYLAIRPGVVIGYARNEKTNEALKDAGITVLPFKGNQLSLGMGNARCMSMPLSRKDVKW

SEQ ID NO: 32 - protein, 411 aa, Mycoplasma spumans
MSVFDSKFKGIHVYSEIGELESVLVHEPGREIDYITPARLDELLFSAILESHDARKEHKGFVAELKKQNVNVIELTDLVAETYELASKEAQAKLIEDFIEDSEPVLNAEEAQAVRKFLSERKSTREMVEYMMSGLTKYELGLESADRELIVDPMPNLYFTRDPFASVGNGVTIHYMKYKVRQRETLFAKFVFSNHPKLVNTPRYYDPSMKLPIEGGDVFIYNNETLVVGCSERTELETITLLAKNIKANKEVEFKRIVAINVPKWTNLMHLDTWLTMLDKDKFLYSPIANDVFKFWDYDLVNGGEEPQPVENGLPLEELLASIINKKPTLIPIAGEGATHIDVERETHFDGTNYLAIAPALIIGYSRNEKTNAALEKAGITVLPFHGNQLSLGMGNARCMSMPLSRKDVKW

SEQ ID NO: 33 - protein, 410 aa, Mycoplasma auris
MSVFDSKFKGIHVYSEIGELETVLVHEPGREIDYITPKRLDELLFSAILESHEARKEHKQFVAELKANDINVVELTDLVAETYDLVSQELKDKLIEEFLDDSYPVLTEEHKKAVRSFLKSRSSTRELIEYMMAGITKYDLGIEAEGDLIVDPMPNLYFTRDPFASVGNGVTIHYMRYKVRQRETLFSRFIFDNHPKLVNTPRYYDPSLKLSIEGGDVFIYNNDTLVMGVSERTDLETVTLLAKNIVANKECEFKRIVAINVPHWTNLMHLDTWLTMLDKDKFLYSPIANDYFKFWDYDLVNGGAEPQPVVNELPLDKLLESIIHKKPILIPIAGEGASQIDLERETHFDGTNYLVLRPGVVVGYARNEKTNAALEAVGIKVLPFYGNQLSLGMGNSRCMSMPLSRKDVKW

SEQ ID NO: 34 - protein, 410 aa, Mycoplasma hyosynoviae
MSVFNSKFKGIHVYSEIGDLESVLVHEPGKEIDYITPSRLDELLFSAILESNDARKEHKEFVEILKKEGVNVVELVDLIAETIDLVDAKKKEALIDEYIEDSEPVVDAKVKPLVKKLLLGIKDTKELVKLMMAGITKYDLEIESEKELIIDPMPNLYFTRDPFASVGNGVTIHYMRYKVRQRETLFSRFVFRNHPKLTSTPWYYDPAMKLSIEGGDVFIYNNDTLVVGVSERTDLDTITLLAKNIKANKECEFKRIVAINVPKWTNLMHLDTWLTMLDKDKFLYSPIANDIFKFWDYDLVNGGSEPQPKDNGLPLEKLLESIIGKKPVLIPIAGCCASDIEIARETHFDGTNYLAIKPGVVIGYARNEKTNKALEKAGIKVLPFKGNQLSLGMGNARCMSMPLSRKDVKW

SEQ ID NO: 35 - protein, 409 aa, Mycoplasma cloacale
MSVFDKRFKGIHVYSEIGELQTVLVHEPGREIDYITPARLDELLFSAILESHDARKEHKEFVKILESQGINVVELTDLIAETYELASEEAKDNLIEEFLDESEPVLSEEHRILVRNFLKGITKTKELVKMMMAGITKYDLGIEADRELIVDPMPNLYFTRDPFASVGNGVTIHYMRYKVRQRETLFSRFIFENHPKLVSTPIYYHPSQGLSIEGGDVFIYNNDTLVVGVSERTDLQTITLLAKNIKANEECEFKRIVAINVPKWTNLMHLDTWLTMLDKNKFLYSPIANDVFKFWDYDLVNGGDEPQPVDNGLPLNELLASIIGEEPVLVPIAGEGASKMDIERETHFDGTNYLAIAPGVVVGYSRNEKTNAALEKAGIKVLPFKGHQLSLGMGNARCMSMPLYRKDVK

SEQ ID NO: 36 - protein, 412 aa, Mycoplasma alkalescens
MSVFDSKFKGIHVYSEIGELESVLVHEPGHEIDYITPSRLDELLFSAMLESHDARKEHKQFVAELKANNVNVIELTDLVAETYDLASQEAKDKLIEEFLEDSEPVLSEENKIAVRDFLKSRKTTRELIEVMMAGITKYDLGIKNCKCQDLVVDPMPNLYFTRDPFASVGNGITIHYMRYKVRQRETLFSRFIFANHPKLVNTPIYYHPSLKLSIEGGDVFIYNNDTLVVGVSERTDLETITLLAKNIVANKECEFKRIVAINVPKWTNLMHLDTWLTMLDKDKFLYSPIANDVFKFWDYDLVNGGAEPKPVENGSSLEAILESIIHKKPILIPIGGDSASQIEVERETHFDGTNYLAIRPGVVIGYSRNVKTNAALEAAGIKVIPFHGNQLSLGMGNARCMSMPLSRKDVKW

SEQ ID NO: 37 - protein, 401 aa, Mycoplasma iners
MSKINVYSEIGVLKEVLVHTPGDEIRRIAPSRLDELLFSAILEPSAAIQEHKSFLKILQDRGIKTIQLSDLVAETYKHYASEAEKEAFIEKYLDEATPVLSKDMRAKVKNYILSMQGEPVKMVRTMMAGVSKQELNVESEVELIVDPMPNLYFTRDPFASAGNGISLNNMKYVVRKRETIFAEFIFSIHPEYKKTPHWFDRLDNGSIEGGDVFIYNKDTLVIGVSERTNKEAIITIAKHIQDNKEAQFKKIVAINVPPMPNLMHLDTWLTMVDKNKFLYSPNMLSVLKVWEIDLSKPIEMVETNKPLAEVLESIIGEKPILIPIAGKDATQLDIDIETHFDGTNYLTIAPGVVVGYSRNVKTEAALRAAGVTVLSFEGNQLSLGMGSARCMSMPLVREDVK

SEQ ID NO: 38 - protein, 401 aa, Mycoplasma gallinarum
MSKIRVYSEIGNLKKVLVHTPGDEIRRISPSRLEELLFSAVLEPNAAIEEHKRFVKLLEDRGIQAIQLSDLVAETYVKYATAEQKAAFIEKYLDEATPALSAENRERAKKYILSLEMQPVKMIRTMMAGLSKYELNVESNIELIIDPMPNLYFTRDPFASAGNGISLNNMKYVVRKRETIFAEFIFAIHPEYKETPHWFDRLDHGSIEGGDVFVYNKDTLVIGVSERTNKEAIITIAKHIQDNKEAEFKKIVAINVPPMPNLMHLDTWLTMVDKNKFIYSPNMLSVLKIWEIDLAKPIEMVESNKSLTEVLESIIGEKPILIPIAGEGASQLDIDIETHFDGTNYLTIAPGVVVGYSRNEKTEKALKAAGITVLSFEGNQLSLGMGSARCMSMPLVREDVK

SEQ ID NO: 39 - protein, 405 aa, Mycoplasma pirum
MNSNQKGIHVYSEIGKLKEVLVHRPGRELDFLDPTRLDELLFAATLEAETARLEHDNFTNALKNQGVTVIELADLVAQTYSSSTPTIKAAFINKYLDEATPALTTKLRTLVKDFLTKQKSVRKMVDYMIGGILSTDLNIKGKPELIVEPMPNAYFTHDPFASVGNGVTLHYMKHNVRRREVLFSEFIFNNNERFQNTPRYIVPTKGLDIEGGDVFVYNKNTLVVGVSERTKMVTIKELAKNILKNKECLFKKIYAINVPKMPNLMHLDTWLTMLDHNKFLYSPNMLSVLKIWEIDISSGKSISSPKELNMDLSKALSIIIGKKPILIPVAGENASQIDINIETNFDATNYLVTQPGVVVGYSRNKKTEAALIKAGIEVIPFQGNQLSLGMGSARCMSMPLIREDV

SEQ ID NO: 40 - protein, 404 aa, Mycoplasma primatum
MSKSKINVYSEYGNLKEVLVHTPGDEIRRITPSRLDELLFSAILEPKSAIAEHKSFCQILKDNKVKAIQLDELVAATYKGVSESVQNSFVERWLDECEPKLENNVRPIVKEYLLKAAEQSVKKMIRIMMAGIDKREIGVESEVDFIVDPMPNLYFTRDPFASVGNGITLHHMKYVVRQRETLFSEFIFDNHPDYKFVPRYFDRDDEGKIEGGDVFIYNSKTLVVGISERTNKDAIRIVAKKIQANADAKFEKIFAINVPPMPNLMHLDTWLTMLDSNKFLYSPNMLSVLKVWEINLDDPALEWKEISGSLEEILTYIIGKKPILIPIAGKGASQFEIDIETHFDGTNYLAIAPSVVIGYSRNELTEKALKKAGVKVLSLDGNQLSLGMGSARCMSMPLIREDVK

SEQ ID NO: 41 - protein, 401 aa, Mycoplasma lipofaciens
MSKINVYSEVGVLKEVLVHTPGDEIRRVAPSRLDELLFSAILEPQDAIAEHKRFIKILEDNNIKVIQLDELVSETWEKATAEQRDAFIEKWLDEAEPVLDAKLRETVKKYLLSLNPVKKMVRTMMAGIDKKELKIELDRDLVVDPMPNLYFTRDPFASAGNGISLNNMKYVTRKRETIFAEFIFNIHPDYKTTPHWFDRLDKGNIEGGDVFIYNKDTLVLGVSERTNKDAVMTIAKHIQSNEQAKFKKLVAINVPPMPNLMHLDTWLTMVDHDKFLYSPNMLSVLKIWEIDLTPGKEIEMVESTKSLSDMLESIIGKKPVLIPIAGKDASQLDIDIETHFDGTNYLTIRPGVVVGYSRNCLTEQALKDAGVTVLSFDGNQLSLGMGSARCMSMPLVREDIK

SEQ ID NO: 42 - protein, 405 aa, Mycoplasma felifaucium
MNKINVYSEIGKLKEVLVHTPGNEIRRISPSRLDELLFSALLEPNFAAKEHTAFCEILKENGIKAIQLVDLVSDTWRIASEKAKTEFIERWLDECEPKLDSNLREIVRKHIYAIEKRSVKRMVKTMMAGIERRELPVTSKEVARELVVDPMPNLYFTRDPFASVGNGISLHHMKYVTRQRETIFAEFVFGNHPDYIDTPRWFDRSDDGRIEGGDVFIYGSKTLVIGVSERTNKEAIKVMAKKIQANKEATFEKIYAINVPPMPNLMHLDTWLTMLDKNKFLYSPNMLAVLQVWEIDLKDPELTWHELSGSLEEILHKIIGRKPILIPIAGHGAQQIDIDIETHFDGTNYLAIAPGVVVGYNRNVLTERALKKAGIKVLSFEGNQLSLGMGSARCMSMPLIRENLK

SEQ ID NO: 43 - protein, 404 aa, Mycoplasma imitans
MFNKIKVYSEIGRLRKVLVHTPGKELEYVTPQRLDELLFSSLLNPVKARQEHEAFIKILQDQGVECVQLTTLTAQTFQSATSEVKEKFINRWLDECLPKLSDDNRIKVYAYLKDLSSDPEVMIRKMMSGILAKEVNVQSDVELIADPMPNLYFTRDPFASIGKGVTLHSMFHPTRKRETIFADFVFSHHPEYKQTPKYYSRLNEYSIEGGDLFVYDDKTLVIGVSERTEKKAIQFLAEKLRENYETTFEKIYAINVPKMSNLMHLDTWLTMLDYDKFLYSPNMMGVLKIWEIDLTHEQLSWRELNESLEEFLSMVIGKKATTIPVAGEDSTQIEIDVETNFDATNFLVIQPGVVVGYDRNYKTNQALVNAGIKVLSWNGDQLSLGMGSARCMSMPLYRDPIKKG

SEQ ID NO: 44 - protein, 401 aa, Mycoplasma opalescens
MSKINVYSEIGTLKEVLVHTPGDEIRRVAPARLDELLFSAILEPNHAIAEHKAFIKILEDNGIKVIQLDELVVQTWNQVDEATRKAFVTKWLDECEPKLESNVRVEVEKYIYSLAKEPKKMVRTMMAGISKEELPLNVNRPLVVDPMPNLYFTRDPFASVGTGISLHHMKYVTRQRETIFAQFVFDNHKDYNTVPRWFDNKDQGRIEGGDVFIYNTKTLVIGVSERTDKDAIKIMAKKIQADKNCKFEKIFAINVPPMPNLMHLDTWLTMVDRNKFLYSPNMLSVLKVWEIDLKDASLAWKEIEGSLSQILEKIIGEKPILIPIAGENASQLDIDIETHFDGTNYLTIAPGVVVGYSRNVKTEQALKAAGVKVLSFEGNQLSLGMGSARCMSMPLIREDLK

SEQ ID NO: 45 - protein, 425 aa, Mycoplasma moatsii
MKKNAINVYSEIGKLKKVLVHRPGDELKYVTPQRMDELLMSAIIELEQAKEEHDAFTKILRDNGVEVIELADLTAEMYDSLTPSEKDAFLNQWVKEASWGKKSSIDALKIKKNLSKKVFDYVKSIKPTRKMIDKLMAGVLLSEIGEKSIILNKDKKNEMVIDLVVDPMPNLYFTRDPFASVGNGITLHNMKYPTRKRETIFAQWIFNKHPEYKDVPQFISKRDGKETIEGGDVFIYTKDVLAIGVSERTNMEAILRIATNIKKDKNCEFKKIVAINVPPMGNLMHLDTWLTMLDKDLFLYSGNIKSALKVWEIDLTKPITPKSPKLSTAKLADILAKIVGKKVRMIPIGGKDGNQMDIDIETHFDGTNYLAIAPGVVVGYHRNRKTQKALEEAGVKVLAFQGNQLSLGMGSARCMSMPLVREEVK

SEQ ID NO: 46 - protein, 399 aa, Mycoplasma elephantis
MSQINVFSEIGQLKEVLVHTPGDEIRRISPKRYNELLFSAILEADVAIKEHKSFVKILEENNVKVIQLKDILLETWNICSKEAKNIFINKWIEEAQPVIHSSSLKEKIKLFLKSKTPLEIIDIMMKGILKQELGIEYKHELIIDPMPNLYFTRDPFTSMGSGITINNMKYQTRKRETIFSEFIFNNHPKYKNTPRWFDRFDSGNIEGGDLFVYTKETIVVGVSERTKKKAILKIAKNIQENNNSFKKIVVIKVPIMQNLMHLDTWIVMVDFDKFIYSPNVTKSLKFWEIDLTKKPKFIQLKNETLEDVLYRVIGKKPILIPVAGENANQIDIDVETHFDATNYLTIRPGVVVGYSRNKKTEEALINAGVKVYAFEGNQLSLGMGSARCMSMPLIREDII

SEQ ID NO: 47 - protein, 399 aa, Mycoplasma testudinis
MKNINVYSEVGKLKEVVVHTPGEELHNVAPSRLQELLTSAVLEPEVARKEHLKFIKILNDYGVKVIQIVDLITETYEAVDSNKKEAFINNWLDNSVPKLTDKNRMILRNYLTQFSTKAMIRKMISGIRAKELNLKTPSALLVDPMPNLCFARDTFACVGSAISLSTMKHPTRRREALLTEFIFQNHPKYKDVIKYFDSKNSKATIEGGDIFVYNPKTLVVGNSERTNMQACLLLAKKIQSNPNNKFEKIVIVNVPPLPHLMHLDTWLTMVDYDKFIYSPNILHTLKFWVIDLKKRKLEAVEKHNTLKAMLRMIIKKEPILIPVGDVGADQLDIDLETHFDATNYLALAPGVVVGYDRNIKTQRALEKAGVKVLSFSGNQLSLAMGSARCLSMPLIREEN

SEQ ID NO: 48 - protein, 410 aa, Mycoplasma canadense
MSVFDSKFKGIHVYSEIGELESVLVHEPGREIDYITPARLDELLFSAILESHDARKEHKQFVSELKANDINVVELTDLVAETYDLASQEAKDKLIEEFLEDSEPVLSEEHKAIVRKYLKGIQPTRKLIEMMMAGITKYDLGIEADHELIVDPMPNLYFTRDPFASVGNGVTIHYMRYKVRQRETLFSRFVFSNHPKLVNTPWYYDPSLKLSIEGGDVFVYNNDTLVVGVSERTDLQTVTLLAKNIVANKECEFKRIVAINVPKWTNLMHLDTWLTMLDKDKFLYSPIANDVFKFWDYDLVNGGSEPQPVENGLPLEGLLESIINKKPILIPIAGEGASQMEIERETHFDGTNYLAIRPGVVIGYSRNEKTNAALEAAGIKVLPFHGNQLSLGMGNARCMSMPLSRKDVKW

SEQ ID NO: 49 - protein, 409 aa, Mycoplasma anseris
MSVFDKRFKGIHVYSEIGELQTVLVHEPGREIDYITPARLDELLFSAILESHDARAEHKKFVATLKEQGINTVELTDLVAETYDLASQEARDNLLEEFLDDSAPVLSEEHKEIVRTYLKGIKGTRKLIETMMAGITKYDLGIEAEQELIVDPMPNLYFTRDPFASVGNGVTIHYMRYKVRQRETLFSRFIFSNHPQLVNTPWYYNPAEGLSIEGGDVFIYNNDTLVVGVSERTDLQTITLLAKNIKANEECEFKRIVAINVPKWTNLMHLDTWLTMLDTNKFLYSPIANDVFKFWDYDLVNGGDEPQPVDNGLPLNELLKSIIGEEPILIPIAGDGATQIEIERETHFDGTNYLAIAPGVVIGYSRNEKTNAALEAAGIKVLPFKGHQLSLGMGNARCMSMPLYRKDVK

SEQ ID NO: 50 - protein, 401 aa, Mycoplasma meleagridis
MSKINVYSEIGVLKEVLVHTPGDEIRRISPSRLDELLFSAILQPEQAIKEHQSFVKILQDRGIKVIQLSDLVAETYVKYATSKEKESFIEKWLDEATPALNSENRARVKNYITAMQGQPVKMVRAMMAGVSKQELNIESDVELIVDPMPNLYFTRDPFASAGNGISLNNMKYVVRKRETIFAEFIFSIHPEYKQTPHWFDRLDKGNIEGGDVFIYNKDTLVIGVSERTNKEAILTIAEHIKNNKEAKFKKIVAINVPPMPNLMHLDTWLTMVDKNKFLYSPNMLSVLKIWEIDLSKEIKMVETSKPLADVLESIIGEKPILIPIAGENASQLDIDIETHFDGTNYLTIAPGVVVGYSRNVKTEAALKAAGVTVYSFDGNQLSLGMGSGRCMSMPLVREDVK

SEQ ID NO: 51 - protein, 404 aa, Mycoplasma alvi
MSIKENGIHVYSEIGKLRDVLVHRPGRELNFLDPSRLDELLFAATLEPETARLEHDNFTTVLKNQGVNVIELADLVSQTYSKVDSKVKKEFIDQYLNEATPKLTSELSKKVYDFLTKQKSNREMVDFMMGGILSSDLNIKGQPYLIVEPMPNLYFTRDPFASVGNGATIHWMKHNVRRREVLFANFIFKYNERFQNTPKYITPTKGLDIEGGDVFVYNKKTLVVGVSERTKMETIKELAKNISKNKECTFTKIYAINVPKMPNLMHLDTWLTMLDYNKFLYSPNMLSVLKVWEINISNNKVSAPKELNVNLEKALSMIIGKKPILIPVAGANASQIDINIETNFDATNYLVIEPGVVVGYSRNKKTEEALVKAGIKVLPFHGNQLSLGMGSARCMSMPLYREDV

SEQ ID NO: 52 - protein, 410 aa, Mycoplasma penetrans
MSSIDKNSLGNGINVYSEIGELKEVLVHTPGDEIRYTAPSRLEELLFSAVLKADTAIEEHKGFVKILQNNGIKVIQLCDLVAETYELCSKEVRNSFIEQYLDEALPVLKKEIRPVVKDYLLSFPTVQMVRKMMSGILANELNIKQDNPLIIDGMPNLYFTRDPFASMGNGVSINCMKYPTRKREVIFSRFVFTNNPKYKNTPRYFDIVGNNGTIEGGDIFIYNSKTLVIGNSERTNFAAIESVAKNIQANKDCTFERIVVINVPPMPNLMHLDTWLTMLDYDKFLYSPNMMNVLKIWEIDLNVKPVKFVEKKGTLEEVLYSIIDKKPILIPIAGKGANQLDIDIETHFDGTNYLTIAPGVVVGYERNEKTQKALVEAGIKVLSFNGSQLSLGMGSARCMSMPLIRENLKK

SEQ ID NO: 53 - protein, 404 aa, Mycoplasma fermentans
MKKINVYSEYGKLKEVLVHTPGDEIRRIAPSRLDELLFSAILEPDSAIAEHKRFVQLLKDNGIKVIQLDELFAKTFDLVSESVKQSFIERWLDECEPKLDATLRAKVKEYILELKAKSSKKMVRVMMAGIDKKELGIELDRDLVVDPMPNLYFTRDPFASVGNGISLHHMKYVTRQRETIFSEFIFDNNLDYNTVPRWFDRKDEGRIEGGDVFIYSADTLVVGVSERTNKEAINVMARKIAADKEVKFKRIYAINVPPMPNLMHLDTWLTMLDKNKFLYSPNMLSVLKVWRIDLNDPDFVWHEIEGSLEEILEQIIGMKPILIPIAGKGASQLDIDIETHFDGTNYLTIAPSVVVGYSRNEKTEKALKAAKVKVLSFEGNQLSLGMGSARCMSMPLIREDIKKK

SEQ ID NO: 54 - protein, 404 aa, Mycoplasma pneumoniae
MKYNINVHSEIGQLQTVLVHTPGNEIRRISPRRLDDLLFSAVIEPDTAIQEHQTFCQLLQEQNIEVVQLTDLTATTFDKANATAQNQFIETWLDQAEPKLTPEHRKVAKQYLLEQKAKSTLSMVRSMMGGIDKRKVAAANTINGDFLVDPMPNLYFTRDPFASIGHGISINRMKYLTRRRETLFASFIFANHPIIAARKFYFKPIDMGTIEGGDIFVYDQQTVVMGLSERTTEAAINVLAKKIQQDSSTSFKRIFVINVPQLPNLMHLDTWLTMLDRNKFLYSPNMLAVLKAWRIDFTDPALKWNEIAGDLSTILHTIIGQKPMLIPIAGADANQTEIDIETHFDGTNYLTIAPSVVVGYARNKLTHQTLEAAGVKVIAFKGNQLSLGMGSARCMSMPLVRKPL

SEQ ID NO: 55 - protein, 414 aa, Mycoplasma sp. CAG:877
MEKIHVTSEIGPLKKVLLHRPGNELLNLTPDTLSRLLFDDIPYLPDAIKEHDEFADALRANGVEVVYLENLMADVLDLSDEIRDKFIKQFIYEAGIRTPKYKYLVFDYLDQITNSKKLVLKTMEGIQISDIPRRKREIEKSLVDLIETEDEFIADPMPNLYFTRDPFASVGEGISLNKMYSVTRNRETIYAEYIFKYHPDYKDQARLYYDRYNPYHIEGGDVLNINDHVLAIGISQRTTAEAIDQIAKNLFKDPECKIDTILAFNIPESRAFMHLDTVFTQVDYDKFTYHPGIMGTLQVFEITEGDDPNSDEDLTVTEINAPLEEILTKYVGRKVTLIPCAGGDKVSAEREQWNDGSNTLCIAPGVVVVYDRNNLTNAVLRSYGLKVIEIHGAELSRGRGGPRCMSMPLVREDI

SEQ ID NO: 56 - protein, 408 aa, Mycoplasma sp. CAG:472
MHVTSEIKKLKKVLVHRPGKELLNLTPDTLGRLLFDDIPYLKDAILEHDEFCQILRDNDVEVVYLEDLMAETLDENPQVKPSFIRQFIYEAGVRTPKYKDLLFDYLMSYTNNKELVLKTMEGIKVSEVHRNKQDSEYSLVDQISEETKFLAEPMPNLYFTRDPFASVGDGIILNKMHSVTRSRETIYAYYIFNYHPDYMDKVPKYYDRENPFSIEGGDVLNLNEHTLAIGISQRTSAEAIDLVAKNMFNDEKCNIDTILAFKIPECRAFMHLDTVFTQIDIDKFTYHPGIMDTLEVFEITKNEDDLDEVRVIKKEGSLENILEEYLGIDITLIPCAGGDKIASEREQWNDGTNTLCIAPGVVVVYNRNNITNEVLREKGIKVIEMNSAELSRGRGGPRCMSMPLERED